European Patent Specification EP 4 077 720 B1, published October 9, 2024. Title: MULTIPLEXED ASSAY USING DIFFERENTIAL FRAGMENT SIZE TO IDENTIFY CANCER SPECIFIC CELL-FREE DNA. Applicant: CADEX GENOMICS, CORP. The sequence listing filed with the application follows.

SEQUENCE LISTING (92 sequences)

SEQ ID NO: 1 - DNA, 20 bp, Artificial Sequence
  Description of Artificial Sequence: Synthetic primer
ggaagcggagcttgcagtga

SEQ ID NO: 2 - DNA, 22 bp, Artificial Sequence
  Description of Artificial Sequence: Synthetic primer
agacggagtctcgctctgtcgc

SEQ ID NO: 3 - DNA, 25 bp, Artificial Sequence
  Description of Artificial Sequence: Synthetic probe
agattgcgccactgcagtccgcagt

SEQ ID NO: 4 - DNA, 19 bp, Artificial Sequence
  Description of Artificial Sequence: Synthetic primer
cttgcagtgagccgagatt

SEQ ID NO: 5 - DNA, 21 bp, Artificial Sequence
  Description of Artificial Sequence: Synthetic primer
gagacggagtctcgctctgtc

SEQ ID NO: 6 - DNA, 22 bp, Artificial Sequence
  Description of Artificial Sequence: Synthetic probe
actgcagtccgcagtccggcct

SEQ ID NO: 7 - DNA, 18 bp, Artificial Sequence
  Description of Artificial Sequence: Synthetic primer
gtggctcacgcctgtaat

SEQ ID NO: 8 - DNA, 20 bp, Artificial Sequence
  Description of Artificial Sequence: Synthetic primer
gggtttcaccttgttagcca

SEQ ID NO: 9 - DNA, 21 bp, Artificial Sequence
  Description of Artificial Sequence: Synthetic probe
tggatcatgaggtcaggagat

SEQ ID NO: 10 - DNA, 22 bp, Artificial Sequence
  Description of Artificial Sequence: Synthetic primer
aggcaggagaatggcgtgaacc

SEQ ID NO: 11 - DNA, 22 bp, Artificial Sequence
  Description of Artificial Sequence: Synthetic primer
agacggagtctcgctctgtcgc

SEQ ID NO: 12 - DNA, 25 bp, Artificial Sequence
  Description of Artificial Sequence: Synthetic probe
agattgcgccactgcagtccgcagt

SEQ ID NO: 13 - DNA, 19 bp, Artificial Sequence
  Description of Artificial Sequence: Synthetic primer
agaccatcctggctaacaa

SEQ ID NO: 14 - DNA, 17 bp, Artificial Sequence
  Description of Artificial Sequence: Synthetic primer
gccattctcctgcctca

SEQ ID NO: 15 - DNA, 21 bp, Artificial Sequence
  Description of Artificial Sequence: Synthetic primer
tggatcatgaggtcaggagat

SEQ ID NO: 16 - DNA, 19 bp, Artificial Sequence
  Description of Artificial Sequence: Synthetic primer
ccgagtagctgggactaca

SEQ ID NO: 17 - DNA, 26 bp, Artificial Sequence
  Description of Artificial Sequence: Synthetic probe
accatcctggctaacaaggtgaaacc

SEQ ID NO: 18 - DNA, 21 bp, Artificial Sequence
  Description of Artificial Sequence: Synthetic primer
atcctggctaacaaggtcaaa

SEQ ID NO: 19 - DNA, 17 bp, Artificial Sequence
  Description of Artificial Sequence: Synthetic primer
cgggttcacgccattct

SEQ ID NO: 20 - DNA, 20 bp, Artificial Sequence
  Description of Artificial Sequence: Synthetic primer
aatggcggctttgtggaata

SEQ ID NO: 21 - DNA, 25 bp, Artificial Sequence
  Description of Artificial Sequence: Synthetic primer
gtctcccatgtctacttctttctac

SEQ ID NO: 22 - DNA, 24 bp, Artificial Sequence
  Description of Artificial Sequence: Synthetic probe
agaaatcggatggttgccgtgtct

SEQ ID NO: 23 - DNA, 20 bp, Artificial Sequence
  Description of Artificial Sequence: Synthetic primer
aaccctgtgctctctgaaac

SEQ ID NO: 24 - DNA, 17 bp, Artificial Sequence
  Description of Artificial Sequence: Synthetic primer
acgctgccttcaagcat

SEQ ID NO: 25 - DNA, 20 bp, Artificial Sequence
  Description of Artificial Sequence: Synthetic primer
gcccaacagctcattgagaa

SEQ ID NO: 26 - DNA, 18 bp, Artificial Sequence
  Description of Artificial Sequence: Synthetic primer
acggcaaccatccgattt

SEQ ID NO: 27 - DNA, 21 bp, Artificial Sequence
  Description of Artificial Sequence: Synthetic primer
tgtccactcagggttaaatgg

SEQ ID NO: 28 - DNA, 25 bp, Artificial Sequence
  Description of Artificial Sequence: Synthetic primer
gattagggattggtgataactctta

SEQ ID NO: 29 - DNA, 26 bp, Artificial Sequence
  Description of Artificial Sequence: Synthetic probe
aagggcggtgcaagatgtgctttgtt

SEQ ID NO: 30 - DNA, 21 bp, Artificial Sequence
  Description of Artificial Sequence: Synthetic primer
tgtgtccactcagggttaaat

SEQ ID NO: 31 - DNA, 23 bp, Artificial Sequence
  Description of Artificial Sequence: Synthetic primer
gattagggattggtgatgactct

SEQ ID NO: 32 - DNA, 26 bp, Artificial Sequence
  Description of Artificial Sequence: Synthetic probe
aagggcggtgcaagatgtgctttgtt

SEQ ID NO: 33 - DNA, 18 bp, Artificial Sequence
  Description of Artificial Sequence: Synthetic primer
tgtgcccaacagctcatt

SEQ ID NO: 34 - DNA, 18 bp, Artificial Sequence
  Description of Artificial Sequence: Synthetic primer
acggcaaccatccgattt

SEQ ID NO: 35 - DNA, 23 bp, Artificial Sequence
  Description of Artificial Sequence: Synthetic primer
ctgtgtccactcagggttaaatg

SEQ ID NO: 36 - DNA, 27 bp, Artificial Sequence
  Description of Artificial Sequence: Synthetic primer
attacttgagattagggattggtgatg

SEQ ID NO: 37 - DNA, 26 bp, Artificial Sequence
  Description of Artificial Sequence: Synthetic probe
aagggcggtgcaagatgtgctttgtt

SEQ ID NO: 38 - DNA, 21 bp, Artificial Sequence
  Description of Artificial Sequence: Synthetic primer
cccaacagctcattgagaacg

SEQ ID NO: 39 - DNA, 21 bp, Artificial Sequence
  Description of Artificial Sequence: Synthetic primer
ctttctacacagacacggcaa

SEQ ID NO: 40 - DNA, 22 bp, Artificial Sequence
  Description of Artificial Sequence: Synthetic primer
ctctctgaaacatgtgctgtgt

SEQ ID NO: 41 - DNA, 23 bp, Artificial Sequence
  Description of Artificial Sequence: Synthetic primer
gggattggtgatgactcttaacg

SEQ ID NO: 42 - DNA, 26 bp, Artificial Sequence
  Description of Artificial Sequence: Synthetic probe
aagggcggtgcaagatgtgctttgtt

SEQ ID NO: 43 - DNA, 22 bp, Artificial Sequence
  Description of Artificial Sequence: Synthetic primer
ctgtgtccactcagggttaaat

SEQ ID NO: 44 - DNA, 25 bp, Artificial Sequence
  Description of Artificial Sequence: Synthetic primer
tgattacttgagattagggattggt

SEQ ID NO: 45 - DNA, 26 bp, Artificial Sequence
  Description of Artificial Sequence: Synthetic probe
aagggcggtgcaagatgtgctttgtt

SEQ ID NO: 46 - DNA, 22 bp, Artificial Sequence
  Description of Artificial Sequence: Synthetic primer
ctgtgtccactcagggttaaat

SEQ ID NO: 47 - DNA, 25 bp, Artificial Sequence
  Description of Artificial Sequence: Synthetic primer
tgtgtccctgattacttgagattag

SEQ ID NO: 48 - DNA, 22 bp, Artificial Sequence
  Description of Artificial Sequence: Synthetic primer
cctgttgatctgtgaccttacc

SEQ ID NO: 49 - DNA, 17 bp, Artificial Sequence
  Description of Artificial Sequence: Synthetic primer
acgctgccttcaagcat

SEQ ID NO: 50 - DNA, 26 bp, Artificial Sequence
  Description of Artificial Sequence: Synthetic probe
aagggcggtgcaagatgtgctttgtt

SEQ ID NO: 51 - DNA, 20 bp, Artificial Sequence
  Description of Artificial Sequence: Synthetic primer
gttgccgtgtctgtgtagaa

SEQ ID NO: 52 - DNA, 20 bp, Artificial Sequence
  Description of Artificial Sequence: Synthetic primer
tttcagagagcacagggttg

SEQ ID NO: 53 - DNA, 26 bp, Artificial Sequence
  Description of Artificial Sequence: Synthetic probe
aagggcggtgcaagatgtgctttgtt

SEQ ID NO: 54 - DNA, 20 bp, Artificial Sequence
  Description of Artificial Sequence: Synthetic primer
aaccctgtgctctctgaaac

SEQ ID NO: 55 - DNA, 25 bp, Artificial Sequence
  Description of Artificial Sequence: Synthetic primer
gattagggattggtgataactctta

SEQ ID NO: 56 - DNA, 26 bp, Artificial Sequence
  Description of Artificial Sequence: Synthetic probe
aagggcggtgcaagatgtgctttgtt

SEQ ID NO: 57 - DNA, 22 bp, Artificial Sequence
  Description of Artificial Sequence: Synthetic primer
ctgtgtccactcagggttaaat

SEQ ID NO: 58 - DNA, 22 bp, Artificial Sequence
  Description of Artificial Sequence: Synthetic primer
gagggaaggtcagcagataaac

SEQ ID NO: 59 - DNA, 26 bp, Artificial Sequence
  Description of Artificial Sequence: Synthetic probe
aagggcggtgcaagatgtgctttgtt

SEQ ID NO: 60 - DNA, 24 bp, Artificial Sequence
  Description of Artificial Sequence: Synthetic primer
cctgtgctctctgaaacatgtgct

SEQ ID NO: 61 - DNA, 24 bp, Artificial Sequence
  Description of Artificial Sequence: Synthetic primer
gatttggcagggtcatgggacaat

SEQ ID NO: 62 - DNA, 26 bp, Artificial Sequence
  Description of Artificial Sequence: Synthetic probe
aagggcggtgcaagatgtgctttgtt

SEQ ID NO: 63 - DNA, 24 bp, Artificial Sequence
  Description of Artificial Sequence: Synthetic primer
atgtgctgtgtccactcagggtta

SEQ ID NO: 64 - DNA, 24 bp, Artificial Sequence
  Description of Artificial Sequence: Synthetic primer
attcttgggtgtttctcacagagg

SEQ ID NO: 65 - DNA, 26 bp, Artificial Sequence
  Description of Artificial Sequence: Synthetic probe
aagggcggtgcaagatgtgctttgtt

SEQ ID NO: 66 - DNA, 24 bp, Artificial Sequence
  Description of Artificial Sequence: Synthetic primer
tgggatcctgttgatctgtgacct

SEQ ID NO: 67 - DNA, 24 bp, Artificial Sequence
  Description of Artificial Sequence: Synthetic primer
gatttggcagggtcatgggacaat

SEQ ID NO: 68 - DNA, 20 bp, Artificial Sequence
  Description of Artificial Sequence: Synthetic primer
gttgccgtgtctgtgtagaa

SEQ ID NO: 69 - DNA, 20 bp, Artificial Sequence
  Description of Artificial Sequence: Synthetic primer
atgggacaatagtggaggga

SEQ ID NO: 70 - DNA, 24 bp, Artificial Sequence
  Description of Artificial Sequence: Synthetic primer
ccgtgtctgtgtagaaagaagtag

SEQ ID NO: 71 - DNA, 18 bp, Artificial Sequence
  Description of Artificial Sequence: Synthetic primer
gggatttggcagggtcat

SEQ ID NO: 72 - DNA, 19 bp, Artificial Sequence
  Description of Artificial Sequence: Synthetic primer
ggcggctttgtggaataga

SEQ ID NO: 73 - DNA, 22 bp, Artificial Sequence
  Description of Artificial Sequence: Synthetic primer
gagggaaggtcagcagataaac

SEQ ID NO: 74 - DNA, 24 bp, Artificial Sequence
  Description of Artificial Sequence: Synthetic probe
atcagggacacaaacactgcggaa

SEQ ID NO: 75 - DNA, 22 bp, Artificial Sequence
  Description of Artificial Sequence: Synthetic primer
tggaatagaaaggcaggaaagg

SEQ ID NO: 76 - DNA, 20 bp, Artificial Sequence
  Description of Artificial Sequence: Synthetic primer
gcagggtcatgggacaatag

SEQ ID NO: 77 - DNA, 23 bp, Artificial Sequence
  Description of Artificial Sequence: Synthetic primer
cacaatagcaaagacttggaacc

SEQ ID NO: 78 - DNA, 19 bp, Artificial Sequence
  Description of Artificial Sequence: Synthetic primer
cccttcctgtgtccatgtg

SEQ ID NO: 79 - DNA, 28 bp, Artificial Sequence
  Description of Artificial Sequence: Synthetic probe
cctttgtagggacatggatgaaagtgga

SEQ ID NO: 80 - DNA, 21 bp, Artificial Sequence
  Description of Artificial Sequence: Synthetic primer
gacttggaaccaacccaaatg

SEQ ID NO: 81 - DNA, 18 bp, Artificial Sequence
  Description of Artificial Sequence: Synthetic primer
cccagagtgtgacgttcc

SEQ ID NO: 82 - DNA, 26 bp, Artificial Sequence
  Description of Artificial Sequence: Synthetic probe
agtgagaacacatggacacaggaagg

SEQ ID NO: 83 - DNA, 22 bp, Artificial Sequence
  Description of Artificial Sequence: Synthetic primer
gtggcacatatacaccatggaa

SEQ ID NO: 84 - DNA, 26 bp, Artificial Sequence
  Description of Artificial Sequence: Synthetic primer
cgttaggtatatctcccaatgctatc

SEQ ID NO: 85 - DNA, 25 bp, Artificial Sequence
  Description of Artificial Sequence: Synthetic probe
tgagaacacatggacacaggaaggg

SEQ ID NO: 86 - DNA, 20 bp, Artificial Sequence
  Description of Artificial Sequence: Synthetic primer
acttggaaccaacccaaatg

SEQ ID NO: 87 - DNA, 19 bp, Artificial Sequence
  Description of Artificial Sequence: Synthetic primer
cacaacagtccccagagtg

SEQ ID NO: 88 - DNA, 25 bp, Artificial Sequence
  Description of Artificial Sequence: Synthetic probe
tgagaacacatggacacaggaaggg

SEQ ID NO: 89 - DNA, 24 bp, Artificial Sequence
  Description of Artificial Sequence: Synthetic primer
catggaatactatgcagccataaa

SEQ ID NO: 90 - DNA, 21 bp, Artificial Sequence
  Description of Artificial Sequence: Synthetic primer
cccactaactcgtcatctagc

SEQ ID NO: 91 - DNA, 25 bp, Artificial Sequence
  Description of Artificial Sequence: Synthetic probe
tgagaacacatggacacaggaaggg

SEQ ID NO: 92 - DNA, 25 bp, Artificial Sequence
  Description of Artificial Sequence: Synthetic probe
tgaggtcaggagatcgagaccatcc